European Patent Specification EP 3 736 346 B1, published December 20, 2023. Title: METHODS AND COMPOSITIONS FOR DIAGNOSING BACTERIAL VAGINOSIS. Applicant: GEN-PROBE INCORPORATED KING, Joseph J. HALL, Jeff G. GRAHAM, Michael. Application TBA. The sequence listing filed with the application follows.

SEQUENCE LISTING (16 sequences)

SEQ ID NO: 1 - DNA, 1486 bp, Eggerthella uncultured bacterium clone rRNA250
  ref <308>: GenBank / AY959023.1
  ref <309>: 2008-04-17
  ref <313>: (1)..(1486)
cgcccttagagtttgatcctggctcaggatgaacgctggcggcgtgcctaacacatgcaagtcgaacgattaaagcaccttcgggtgtgtatagagtggcgaacgggtgagtaacacgtgaccaacctgcctcttacattgggacaaccaaaagaaattctggctaataccaaatactccgcacatatcacatgatgtatgcgggaaagcttttgcggtaagagatggggtcgcggcccattaggtagacggcggggtagaagcccaccgtgccgatgatgggtagccgggttgagagaccgaccggccacattgggactgagatacggcccagactcctacgggaggcagcagtggggaatattgcgcaatgggggaaaccctgacgcagcaacgccgcgtgcgggatgaaggccttcgggttgtaaaccgctttcagcagggaagacatcgacggtacctgcagaagaagccccggctaactacgtgccagcagccgcggtaatacgtagggggcgagcgttatccggattcattgggcgtaaagcgcgcgcaggcggttgctcaagcggaacctctaatctcggggcttaacctcgagccgggttccgaactggacgactcgagtgcggtagaggcagatggaattcccggtgtagcggtggaatgcgcagatatcgggaagaacaccaacggcgaaggcagtctgctgggccgtcactgacgctgaggcgcgaaagctgggggagcgaacaggattagataccctggtagtcccagccgtaaacgatgagcgctgggtgtgggagattacatcttccgtgccgaagctaacgcattaagcgctccgcctggggagtacggccgcaaggctaaaactcaaaggaattgacgggggcccgcacaagcagcggagcatgtggcttaattcgaagcaacgcgaagaaccttaccagggcttgacatgtaggtgaagcggcggaaacgtcgtggccgaaaggagcctacacaggtggtgcatggctgtcgtcagctcgtgtcgtgagatgttgggttaagtcccgcaacgagcgcaacccctgccccgtgttaccagcatttagttggggactcgcgggggactgccggcgtcaagccggaggaaggcggggatgacgtcaagtcatcatgccccttatgccctgggccgcacacgtgctacaatggccggcacagcgggctgcaacctagcgataggaagcgaatcccgtaaagccggtcccagttcggattggaggctgaaacccgcctccatgaagccggagttgctagtaatcgcggatcagcacgccgcggtgaatgcgttcccgggccttgtacacaccgcccgtcacaccacccgagtcgtctgcacccgaagccgccggccgaacccctttggggacggaggcgtcgaaggtgtggagggtgaggggggtgaagtcgtaacaaggtaaccgtaaagggc

SEQ ID NO: 2 - DNA, 1553 bp, Prevotella bivia
  ref <308>: GenBank / JN867270.1
  ref <309>: 2012-03-30
  ref <313>: (1)..(1553)
tgtgtagcggtgaaatgygtagatatargaaggaacatcagtggcgaaggcgaccacckggwcwgatastgacastgaggtgcgaaagcgtggggagcraacaggattagataccstggtagtccacgccgtaaacgatgtcaacttggctcaggatgaacgctagctataggcttaacacatgcaagtcgaggggcagcgaatagatagcttgctatttatgtcggcgaccggcgcacgggtgagtaacgcgtatccaacctgcccataactaagggataacccagcgaaagttggactaataccttatgtattcgtttgatctcatgagattaygaataaagatttatcggttatggatggggatgcgtctgattagcttgttggcggggtaacggcccaccaaggcaacgatcagtaggggttctgagaggaaggtcccccacattggaactgagacacggtccaaactcctacgggaggcagcagtgaggaatattggtcaatggacgcaagtctgaaccagccaagtagcgtgcaggatgacggcyctatgggttgtaaactgcttttatatggggataaagtggggaacgtgttcccttttgcaggtaccatatgaataaggaccggctaattccgtgccagcagccgcggtaatacggaaggttcgggcgttatccggatttattgggtttaaagggagcgtaggccgtttggtaagcgtgttgtgaaatgtaggagctcaacttctagattgcagcgcgaactgtcagacttgagtgcgcacaacgtaggcggaattcatggtgtagcggtgaaatgcttagatatcatgaagaactccgattgcgaaggcagcttacgggarcgcaactgacgctgaagctcgaaggtgcgggtatcgaacaggattagataccctggtagtccgcacagtaaacgatggatgcccgctgttagcacctagtgttagcggctaagcgaaagcattaagcatcccacctggggagtacgccggcaacggtgaaactcaaaggaattgacgggggcccgcacaagcggaggaacatgtggtttaattcgatgatacgcgaggaaccttacccgggcttgaattgcagatgaacgatttagagataatgaggtccttcgggacatctgtgaaggtgctgcatggttgtcgtcagctcgtgccgtgaggtgtcggcttaagtgccataacgagcgcaacccctttctttagttgccatcaggtymtgctgggcactctggagatactgccaccgtaaggtgtgaggaaggtggggatgacgtcaaatcagcacggyccttacgtccggggctacacacgtgttacaatgggtggtacagatagttggtcgtrtgcaaatacgatctaatccttaaaaccattctcagttcggactggggtctgcaacccgaccccacgaagctggattcgctagtaatcgcgcatcagccatggcgcggtgaatacgttcccgggccttgtacacaccgcccgtcaagccatgaaagccgggggtgcc

SEQ ID NO: 3 - DNA, 2049 bp, Lactobacillus crispatus
  ref <308>: GenBank / FN692037.1
  ref <309>: 2010-06-24
  ref <313>: (1)..(2049)
ttaataaagtcgcttcgagagatgcgacgagagcttaaaaacagacatgtaaggaaagaaaacaaataaaaagaaaaaagtacttgcaaagaagtaaataagctggtaatatatttaaatgtcgtcaggcgaaagcagaaaaagcttgagcaagacgaaaaaaacaaatcaaaaaagttcttgacaaagaaatgatggtttgataaaatataaaagctgtctgctttacaaaaagcaagacagaggtagtactttgaaaactgaacaaagtttcgctaaaagtgtgcgggtgtaaaaacccaaacaagaagcgaagtcaattcgcaagcaataaatttgagacaaagatcttaaataaggaatgagcaatcattcaaactttttaaaatgagagtttgatcctggctcaggacgaacgctggcggcgtgcctaatacatgcaagtcgagcgagcggaactaacagatttacttcggtaatgacgttaggaaagcgagcggcggatgggtgagtaacacgtggggaacctgccccatagtctgggataccacttggaaacaggtgctaataccggataagaaagcagatcgcatgatcagcttttaaaaggcggcgtaagctgtcgctatgggatggccccgcggtgcattagctagttggtaaggtaaaggcttaccaaggcgatgatgcatagccgagttgagagactgatcggccacattgggactgagacacggcccaaactcctacgggaggcagcagtagggaatcttccacaatggacgcaagtctgatggagcaacgccgcgtgagtgaagaaggttttcggatcgtaaagctctgttgttggtgaagaaggatagaggtagtaactggcctttatttgacggtaatcaaccagaaagtcacggctaactacgtgccagcagccgcggtaatacgtaggtggcaagcgttgtccggatttattgggcgtaaagcgagcgcaggcggaagaataagtctgatgtgaaagccctcggcttaaccgaggaactgcatcggaaactgtttttcttgagtgcagaagaggagagtggaactccatgtgtagcggtggaatgcgtagatatatggaagaacaccagtggcgaaggcggctctctggtctgcaactgacgctgaggctcgaaagcatgggtagcgaacaggattagataccctggtagtccatgccgtaaacgatgagtgctaagtgttgggaggtttccgcctctcagtgctgcagctaacgcattaagcactccgcctggggagtacgaccgcaaggttgaaactcaaaggaattgacgggggcccgcacaagcggtggagcatgtggtttaattcgaagcaacgcgaagaaccttaccaggtcttgacatctagtgccatttgtagagatacaaagttcccttcggggacgctaagacaggtggtgcatggctgtcgtcagctcgtgtcgtgagatgttgggttaagtcccgcaacgagcgcaacccttgttattagttgccagcattaagttgggcactctaatgagactgccggtgacaaaccggaggaaggtggggatgacgtcaagtcatcatgccccttatgacctgggctacacacgtgctacaatgggcagtacaacgagaagcgagcctgcgaaggcaagcgaatctctgaaagctgttctcagttcggactgcagtctgcaactcgactgcacgaagctggaatcgctagtaatcgcggatcagcacgccgcggtgaatacgttcccgggccttgtacacaccgcccgtcacaccatgggagtctgcaatgcccaaagccggtggcctaaccttcgggaaggagccgtctaaggcagggcagatgactggggtgaagtcgtaacaaggtagccgtaggagaacctgcggctggatcacctcctttctaaggaagcgaaggatatggagagcaggaatgctaagagaagtatccagagcaagcggaagcacactgagaaactttgtttagttttgagggtagtacctc

SEQ ID NO: 4 - DNA, 27 bp, Artificial Sequence
  Synthetic Oligonucleotide
gactaacaacgaggcagatggaattcc

SEQ ID NO: 5 - DNA, 21 bp, Artificial Sequence
  Synthetic Oligonucleotide
tggacgactcgagtgcggtaa

SEQ ID NO: 6 - DNA, 18 bp, Artificial Sequence
  Synthetic Oligonucleotide
gatatctgcgcattccac

SEQ ID NO: 7 - DNA, 25 bp, Artificial Sequence
  Synthetic Oligonucleotide
gacccttattggctaagcgaaagca

SEQ ID NO: 8 - DNA, 25 bp, Artificial Sequence
  Synthetic Oligonucleotide
ccgctgttagcacctagtgttagca

SEQ ID NO: 9 - DNA, 17 bp, Artificial Sequence
  Synthetic Oligonucleotide
ttgagtttcaccgttgc

SEQ ID NO: 10 - DNA, 27 bp, Artificial Sequence
  Synthetic Oligonucleotide
acagcaaataaggtagtaactggcctt

SEQ ID NO: 11 - DNA, 28 bp, Artificial Sequence
  Synthetic Oligonucleotide
agctctgttgttggtgaagaaggatagc

SEQ ID NO: 12 - DNA, 33 bp, Artificial Sequence
  Synthetic Oligonucleotide
cgtaaagctctgttggtagtgaagaaagatagc

SEQ ID NO: 13 - DNA, 17 bp, Artificial Sequence
  Synthetic Oligonucleotide
tacgtattaccgcggct

SEQ ID NO: 14 - DNA, 34 bp, Artificial Sequence
  Synthetic Oligonucleotide
tcttagccggttttccggctgagagttgttagtc

SEQ ID NO: 15 - DNA, 34 bp, Artificial Sequence
  Synthetic Oligonucleotide
tcttagccggttttccggctgagaaataagggtc

SEQ ID NO: 16 - DNA, 34 bp, Artificial Sequence
  Synthetic Oligonucleotide
tcttagccggttttccggctgagatatttgctgt